European Patent Specification EP 3 833 765 B1, published January 14, 2026. Title: ONCOLYTIC VIRUS CARRYING E-CADHERIN AND USES THEREOF. Applicant: Jianhu YU Michael Caligiuri Bo Xu. The sequence listing filed with the application follows.

SEQUENCE LISTING (3 sequences)

SEQ ID NO: 1 - DNA, 2649 bp, CDS of I cadherin 1 (CDH1) from Homo sapiens cadherin 1 (CDH1), transcript variant 1, mRNA, NCBI Reference Sequence: NM_004360.4 (127..2775)
atgggcccttggagccgcagcctctcggcgctgctgctgctgctgcaggtctcctcttggctctgccaggagccggagccctgccaccctggctttgacgccgagagctacacgttcacggtgccccggcgccacctggagagaggccgcgtcctgggcagagtgaattttgaagattgcaccggtcgacaaaggacagcctatttttccctcgacacccgattcaaagtgggcacagatggtgtgattacagtcaaaaggcctctacggtttcataacccacagatccatttcttggtctacgcctgggactccacctacagaaagttttccaccaaagtcacgctgaatacagtggggcaccaccaccgccccccgccccatcaggcctccgtttctggaatccaagcagaattgctcacatttcccaactcctctcctggcctcagaagacagaagagagactgggttattcctcccatcagctgcccagaaaatgaaaaaggcccatttcctaaaaacctggttcagatcaaatccaacaaagacaaagaaggcaaggttttctacagcatcactggccaaggagctgacacaccccctgttggtgtctttattattgaaagagaaacaggatggctgaaggtgacagagcctctggatagagaacgcattgccacatacactctcttctctcacgctgtgtcatccaacgggaatgcagttgaggatccaatggagattttgatcacggtaaccgatcagaatgacaacaagcccgaattcacccaggaggtctttaaggggtctgtcatggaaggtgctcttccaggaacctctgtgatggaggtcacagccacagacgcggacgatgatgtgaacacctacaatgccgccatcgcttacaccatcctcagccaagatcctgagctccctgacaaaaatatgttcaccattaacaggaacacaggagtcatcagtgtggtcaccactgggctggaccgagagagtttccctacgtataccctggtggttcaagctgctgaccttcaaggtgaggggttaagcacaacagcaacagctgtgatcacagtcactgacaccaacgataatcctccgatcttcaatcccaccacgtacaagggtcaggtgcctgagaacgaggctaacgtcgtaatcaccacactgaaagtgactgatgctgatgcccccaataccccagcgtgggaggctgtatacaccatattgaatgatgatggtggacaatttgtcgtcaccacaaatccagtgaacaacgatggcattttgaaaacagcaaagggcttggattttgaggccaagcagcagtacattctacacgtagcagtgacgaatgtggtaccttttgaggtctctctcaccacctccacagccaccgtcaccgtggatgtgctggatgtgaatgaagcccccatctttgtgcctcctgaaaagagagtggaagtgtccgaggactttggcgtgggccaggaaatcacatcctacactgcccaggagccagacacatttatggaacagaaaataacatatcggatttggagagacactgccaactggctggagattaatccggacactggtgccatttccactcgggctgagctggacagggaggattttgagcacgtgaagaacagcacgtacacagccctaatcatagctacagacaatggttctccagttgctactggaacagggacacttctgctgatcctgtctgatgtgaatgacaacgcccccataccagaacctcgaactatattcttctgtgagaggaatccaaagcctcaggtcataaacatcattgatgcagaccttcctcccaatacatctcccttcacagcagaactaacacacggggcgagtgccaactggaccattcagtacaacgacccaacccaagaatctatcattttgaagccaaagatggccttagaggtgggtgactacaaaatcaatctcaagctcatggataaccagaataaagaccaagtgaccaccttagaggtcagcgtgtgtgactgtgaaggggccgctggcgtctgtaggaaggcacagcctgtcgaagcaggattgcaaattcctgccattctggggattcttggaggaattcttgctttgctaattctgattctgctgctcttgctgtttcttcggaggagagcggtggtcaaagagcccttactgcccccagaggatgacacccgggacaacgtttattactatgatgaagaaggaggcggagaagaggaccaggactttgacttgagccagctgcacaggggcctggacgctcggcctgaagtgactcgtaacgacgttgcaccaaccctcatgagtgtcccccggtatcttccccgccctgccaatcccgatgaaattggaaattttattgatgaaaatctgaaagcggctgatactgaccccacagccccgccttatgattctctgctcgtgtttgactatgaaggaagcggttccgaagctgctagtctgagctccctgaactcctcagagtcagacaaagaccaggactatgactacttgaacgaatggggcaatcgcttcaagaagctggctgacatgtacggaggcggcgaggacgactag

SEQ ID NO: 2 - DNA, 3414 bp, CDS of Human herpesvirus 1 UL39 (ICP6) from Human herpesvirus 1 strain F, complete genome, GenBank: GU734771.1 (86339..89752)
atggccagccgcccagccgcatcctctcccgtcgaagcgcgggccccggttgggggacaggaggccggcggccccagcgcagccacccagggggaggccgccggggcccctctcgcccacggccaccacgtgtactgccagcgagtcaatggcgtgatggtgctttccgacaagacgcccgggtccgcgtcctaccgcatcagcgatagcaactttgtccaatgtggttccaactgcaccatgattatcgacggagacgtggtgcgcgggcgcccccaggacccgggggccgcggcatcccccgctcccttcgttgcggtgacaaacatcggagccggcagcgacggcgggaccgccgtcgttgcattcgggggaaccccacgtcgctcggcggggacgtctaccggtacccagacggccgacgtcccagccgaggcccttgggggcccccctcctcctccccgcttcaccctgggtggcggctgttgctcctgtcgcgacacacggcgccgctctgcggtattcgggggggagggggatcccgtcggccccgcggagttcgtctcggacgaccggtcgtccgattccgactcggatgactcggaggacaccgactcggagacgctgtcacacgcctcctcggacgtgtccggcggggccacgtacgacgacgcccttgactccgattcgtcatcggatgactccctgcagatagatggccccgtgtgtcgcccgtggagcaatgacaccgcgcccctggatgtttgccccgggacccccggcccgggcgccgacgccggtggtccctcagcggtagacccacacgcgccgacgacaggggccggcgctggtcttgcggccgatcccgccgtggcccgggacgacgcggaggggctttcggacccccggccacgtctgggaacgggcacggcctaccccgtccccctggaactcacgcccgagaacgcggaggccgtggcgcgctttctgggagatgccgtgaaccgcgaacccgcgctcatgctggagtacttttgccggtgcgcccgcgaggaaaccaagcgtgtcccccccaggacattctgcagcccccctcgcctcacggaggacgactttgggcttctcaactacgcgctcgtggagatgcagcgcctgtgtctggacgttcctccggtcccgccgaacgcatacatgccctattatctcagggagtatgtgacgcggctggtcaacgggttcaagccgctggtgagccggtccgttcgcctttaccgcatcctgggggttctggtgcacctgcggatccggacccgggaggcctcctttgaggagtggctgcgatccaaggaagtggccctggactttggcctgacggaaaggcttcgcgagcacgaagcccagctggtgatcctggcccaggctctggaccattacgactgtctgatccacagcacaccgcacacgctggtcgagcgggggctgcaatcggccctgaagtatgaggagttttacctaaagcgctttggcgggcactacatggagtccgtcttccagatgtacacccgcatcgccggctttttggcctgccgggccacgcgcggcatgcgccacatcgccctggggcgagaggggtcgtggtgggaaatgttcaagttctttttccaccgcctctacgaccaccagatcgtaccgtcgacccccgccatgctgaacctggggacccgcaactactacacctccagctgctacctggtaaacccccaggccaccacaaacaaggcgaccctgcgggccatcaccagcaacgtcagtgccatcctcgcccgcaacgggggcatcgggctatgcgtgcaggcgtttaacgactccggccccgggaccgccagcgtcatgcccgccctcaaggtcctcgactcgctggtggcggcgcacaacaaagagagcgcgcgtccgaccggcgcgtgcgtgtacctggagccgtggcacaccgacgtgcgggccgtgctccggatgaagggggtcctcgccggcgaagaggcccagcgctgcgacaatatcttcagcgccctctggatgccagacctgtttttcaagcgcctgattcgccacctggacggcgagaagaacgtcacatggaccctgttcgaccgggacaccagcatgtcgctcgccgactttcacggggaggagttcgagaagctctaccagcacctcgaggtcatggggttcggcgagcagatacccatccaggagctggcctatggcattgtgcgcagtgcggccacgaccgggagccccttcgtcatgttcaaagacgcggtgaaccgccactacatctacgacacccagggggcggccatcgccggctccaacctctgcaccgagatcgtccatccggcctccaagcgatccagtggggtctgcaatctgggaagcgtgaatctggcccgatgcgtctccaggcagacgtttgactttgggcggctccgcgacgccgtgcaggcgtgcgtgctgatggtgaacatcatgatcgacagcacgctacaacccacgccccagtgcacccgcggcaacgacaacctgcggtccatgggaatcggcatgcagggcctgcacacggcctgcctgaagctggggctggatctggagtctgccgaatttcaggacctgaacaaacacatcgccgaggtgatgctgctgtcggcgatgaagaccagcaacgcgctgtgcgttcgcggggcccgtcccttcaaccactttaagcgcagcatgtatcgcgccggccgctttcactgggagcgctttccggacgcccggccgcggtacgagggcgagtgggagatgctacgccagagcatgatgaaacacggcctgcgcaacagccagtttgtcgcgctgatgcccaccgccgcctcggcgcagatctcggacgtcagcgagggctttgcccccctgttcaccaacctgtttagcaaggtgacccgggacggcgagacgctgcgccccaacacgctcctgctaaaggaactggaacgcacgtttagcgggaagcgcctcctggaggtgatggacagtctcgacgccaagcagtggtccgtggcgcaggcgctcccgtgcctggagcccacccaccccctccggcgattcaagaccgcgtttgactacgaccagaagttgctgatcgacctgtgtgcggaccgcgccccctacgtcgaccatagccaatccatgaccctgtatgtcacggagaaggcggacgggaccctcccagcctccaccctggtccgccttctggtccacgcatataagcgcggactaaaaacagggatgtactactgcaaggttcgcaaggcgaccaacagcggggtctttggcggcgacgacaacattgtctgcacgagctgcgcgctgtga

SEQ ID NO: 3 - DNA, 747 bp, CDS of Human herpesvirus 1 RL1 (ICP34.5) from Human herpesvirus 1 strain F, complete genome (487..1233) and complement
atggcccgccgccgccgccatcgcggcccccgccgcccccggccgcccgggcccacgggcgccgtcccaaccgcacagtcccaggtaacctccacgcccaactcggaacccgcggtcaggagcgcgcccgcggccgccccgccgccgccccccgccagtgggcccccgccttcttgttcgctgctgctgcgccagtggctccacgttcccgagtccgcgtccgacgacgacgatgacgacgactggccggacagccccccgcccgagccggcgccagaggcccggcccaccgccgccgccccccgcccccggtccccaccgcccggcgcgggcccggggggcggggctaacccctcccaccccccctcacgccccttccgccttccgccgcgcctcgccctccgcctgcgcgtcaccgcagagcacctggcgcgcctgcgcctgcgacgcgcgggcggggagggggcgccggagccccccgcgacccccgcgacccccgcgacccccgcgacccccgcgacccccgcgcgggtgcgcttctcgccccacgtccgggtgcgccacctggtggtctgggcctcggccgcccgcctggcgcgccgcggctcgtgggcccgcgagcgggccgaccgggctcggttccggcgccgggtggcggaggccgaggcggtcatcgggccgtgcctggggcccgaggcccgtgcccgggccctggcccgcggagccggcccggcgaactcggtctaa